European Patent Specification EP 3 686 215 B1, published September 2, 2026. Title: cAMP receptor protein variant and method for producing L-amino acid using the same. Applicant: CJ CheilJedang Corporation. The sequence listing filed with the application follows.

SEQUENCE LISTING (7 sequences)

SEQ ID NO: 1 - protein, 210 aa, Unknown
  CRP
MVLGKPQTDPTLEWFLSHCHIHKYPSKSKLIHQGEKAETLYYIVKGSVAVLIKDEEGKEMILSYLNQGDFIGELGLFEEGQERSAWVRAKTACEVAEISYKKFRQLIQVNPDILMRLSAQMARRLQVTSEKVGNLAFLDVTGRIAQTLLNLAKQPDAMTHPDGMQIKITRQEIGQIVGCSRETVGRILKMLEDQNLISAHGKTIVVYGTR

SEQ ID NO: 2 - DNA, 633 bp, Unknown
  crp
atggtgcttggcaaaccgcaaacagacccgactctcgaatggttcttgtctcattgccacattcataagtacccatccaagagcaagcttattcaccagggtgaaaaagcggaaacgctgtactacatcgttaaaggctctgtggcagtgctgatcaaagacgaagagggtaaagaaatgatcctctcctatctgaatcagggtgattttattggcgaactgggcctgtttgaagagggccaggaacgtagcgcatgggtacgtgcgaaaaccgcctgtgaagtggctgaaatttcgtacaaaaaatttcgccaattgattcaggtaaacccggacattctgatgcgtttgtctgcacagatggcgcgtcgtctgcaagtcacttcagagaaagtgggcaacctggcgttcctcgacgtgacgggccgcattgcacagactctgctgaatctggcaaaacaaccagacgctatgactcacccggacggtatgcaaatcaaaattacccgtcaggaaattggtcagattgtcggctgttctcgtgaaaccgtgggacgcattctgaagatgctggaagatcagaacctgatctccgcacacggtaaaaccatcgtcgtttacggcactcgttaa

SEQ ID NO: 3 - protein, 210 aa, Unknown
  modified CRP
MVLGKPQTDPTLEWFLSHCHIHKYPSKSKLIHQGEKAETLYYIVKGSVAVLIKDEEGKEMILSYLNQGDFIGELGLFEEGQERSAWVRAKTACEVAEISYKKFRQLIQVNPDILMRLSAQMARRLQVTSEKVGNLAFLDVTGRIAQTLLNLAKQPDAMTHPDGMQIKITRQEIGQIVGCSRETVGRILKMLEDQNQISAHGKTIVVYGTR

SEQ ID NO: 4 - DNA, 633 bp, Unknown
  modified crp
atggtgcttggcaaaccgcaaacagacccgactctcgaatggttcttgtctcattgccacattcataagtacccatccaagagcaagcttattcaccagggtgaaaaagcggaaacgctgtactacatcgttaaaggctctgtggcagtgctgatcaaagacgaagagggtaaagaaatgatcctctcctatctgaatcagggtgattttattggcgaactgggcctgtttgaagagggccaggaacgtagcgcatgggtacgtgcgaaaaccgcctgtgaagtggctgaaatttcgtacaaaaaatttcgccaattgattcaggtaaacccggacattctgatgcgtttgtctgcacagatggcgcgtcgtctgcaagtcacttcagagaaagtgggcaacctggcgttcctcgacgtgacgggccgcattgcacagactctgctgaatctggcaaaacaaccagacgctatgactcacccggacggtatgcaaatcaaaattacccgtcaggaaattggtcagattgtcggctgttctcgtgaaaccgtgggacgcattctgaagatgctggaagatcagaaccagatctccgcacacggtaaaaccatcgtcgtttacggcactcgttaa

SEQ ID NO: 5 - DNA, 933 bp, Unknown
  crp and expression control region
tttgctactccactgcgtcaattttcctgacagagtacgcgtactaaccaaatcgcgcaacggaaggcgacctgggtcatgctgaagcgagacaccaggagacacaaagcgaaagctatgctaaaacagtcaggatgctacagtaatacattgatgtactgcatgtatgcaaaggacgtcacattaccgtgcagtacagttgatagccccttcccaggtagcgggaagcatatttcggcaatccagagacagcggcgttatctggctctggagaaagcttataacagaggataaccgcgcatggtgcttggcaaaccgcaaacagacccgactctcgaatggttcttgtctcattgccacattcataagtacccatccaagagcaagcttattcaccagggtgaaaaagcggaaacgctgtactacatcgttaaaggctctgtggcagtgctgatcaaagacgaagagggtaaagaaatgatcctctcctatctgaatcagggtgattttattggcgaactgggcctgtttgaagagggccaggaacgtagcgcatgggtacgtgcgaaaaccgcctgtgaagtggctgaaatttcgtacaaaaaatttcgccaattgattcaggtaaacccggacattctgatgcgtttgtctgcacagatggcgcgtcgtctgcaagtcacttcagagaaagtgggcaacctggcgttcctcgacgtgacgggccgcattgcacagactctgctgaatctggcaaaacaaccagacgctatgactcacccggacggtatgcaaatcaaaattacccgtcaggaaattggtcagattgtcggctgttctcgtgaaaccgtgggacgcattctgaagatgctggaagatcagaacctgatctccgcacacggtaaaaccatcgtcgtttacggcactcgttaa

SEQ ID NO: 6 - DNA, 29 bp, Artificial Sequence
  crp-F
cacgaattctttgctactccactgcgtca

SEQ ID NO: 7 - DNA, 29 bp, Artificial Sequence
  crp-R
acacgaattcttaacgagtgccgtaaacg